European Patent Application EP 4 563 697 A1, published June 4, 2025. Title: In vitro culture method to induce follicle from primate fetal ovarian cell. Applicant: Kyoto University. The sequence listing filed with the application follows.

SEQUENCE LISTING (28 sequences)

SEQ ID NO: 1 - DNA, 20 bp, synthetic construct
  misc_feature 1..20: note = PCR Primer(GAPDH) for Cynomolgus monkey
  source 1..20: mol_type = other DNA
aacagggtggtggacctcat

SEQ ID NO: 2 - DNA, 20 bp, synthetic construct
  misc_feature 1..20: note = PCR Primer(GAPDH) for Cynomolgus monkey
  source 1..20: mol_type = other DNA
ttcctcttgtgctctcgctg

SEQ ID NO: 3 - DNA, 21 bp, synthetic construct
  misc_feature 1..21: note = PCR Primer(NANOG) for Cynomolgus monkey
  source 1..21: mol_type = other DNA
tgttccggtttccattatgcc

SEQ ID NO: 4 - DNA, 20 bp, synthetic construct
  misc_feature 1..20: note = PCR Primer(NANOG) for Cynomolgus monkey
  source 1..20: mol_type = other DNA
taggctccaaccatactcca

SEQ ID NO: 5 - DNA, 20 bp, synthetic construct
  misc_feature 1..20: note = PCR Primer(PPIA) for Cynomolgus monkey
  source 1..20: mol_type = other DNA
acaggtcctggcatcttgtc

SEQ ID NO: 6 - DNA, 20 bp, synthetic construct
  misc_feature 1..20: note = PCR Primer(PPIA) for Cynomolgus monkey
  source 1..20: mol_type = other DNA
ctcagtcttggcagtgcaga

SEQ ID NO: 7 - DNA, 21 bp, synthetic construct
  misc_feature 1..21: note = PCR Primer(DDX4) for Cynomolgus monkey
  source 1..21: mol_type = other DNA
cttcttcagggggcttagaca

SEQ ID NO: 8 - DNA, 24 bp, synthetic construct
  misc_feature 1..24: note = PCR Primer(DDX4) for Cynomolgus monkey
  source 1..24: mol_type = other DNA
actcaagtaaaaatgagacccagt

SEQ ID NO: 9 - DNA, 22 bp, synthetic construct
  misc_feature 1..22: note = PCR Primer(SCP1) for Cynomolgus monkey
  source 1..22: mol_type = other DNA
aggccccttcatctctaacaac

SEQ ID NO: 10 - DNA, 22 bp, synthetic construct
  misc_feature 1..22: note = PCR Primer(SCP1) for Cynomolgus monkey
  source 1..22: mol_type = other DNA
tttagcaattacagcccaacgg

SEQ ID NO: 11 - DNA, 22 bp, synthetic construct
  misc_feature 1..22: note = PCR Primer(ZP3) for Cynomolgus monkey
  source 1..22: mol_type = other DNA
gtccaggtctgcttctcgtaac

SEQ ID NO: 12 - DNA, 22 bp, synthetic construct
  misc_feature 1..22: note = PCR Primer(ZP3) for Cynomolgus monkey
  source 1..22: mol_type = other DNA
ggcccactgctctacttcatag

SEQ ID NO: 13 - DNA, 22 bp, synthetic construct
  misc_feature 1..22: note = PCR Primer(FOXL2) for Cynomolgus monkey
  source 1..22: mol_type = other DNA
ccaccttgggaaggagaaatgt

SEQ ID NO: 14 - DNA, 22 bp, synthetic construct
  misc_feature 1..22: note = PCR Primer(FOXL2) for Cynomolgus monkey
  source 1..22: mol_type = other DNA
ttggtcccccaaacaagttaca

SEQ ID NO: 15 - DNA, 22 bp, synthetic construct
  misc_feature 1..22: note = PCR Primer(GAPDH) for Human
  source 1..22: mol_type = other DNA
acaagaggaagagagagaccct

SEQ ID NO: 16 - DNA, 22 bp, synthetic construct
  misc_feature 1..22: note = PCR Primer(GAPDH) for Human
  source 1..22: mol_type = other DNA
tctacatggcaactgtgaggag

SEQ ID NO: 17 - DNA, 22 bp, synthetic construct
  misc_feature 1..22: note = PCR Primer(NANOG) for Human
  source 1..22: mol_type = other DNA
agaggtctcgtatttgctgcat

SEQ ID NO: 18 - DNA, 22 bp, synthetic construct
  misc_feature 1..22: note = PCR Primer(NANOG) for Human
  source 1..22: mol_type = other DNA
aaacactcggtgaaatcagggt

SEQ ID NO: 19 - DNA, 26 bp, synthetic construct
  misc_feature 1..26: note = PCR Primer(DAZL) for Human
  source 1..26: mol_type = other DNA
gaattcccaagagggctttattacac

SEQ ID NO: 20 - DNA, 27 bp, synthetic construct
  misc_feature 1..27: note = PCR Primer(DAZL) for Human
  source 1..27: mol_type = other DNA
tgatatgtgtcagaatgttatagcacc

SEQ ID NO: 21 - DNA, 26 bp, synthetic construct
  misc_feature 1..26: note = PCR Primer(DDX4) for Human
  source 1..26: mol_type = other DNA
ttgcagttactgatacaaatggtgtt

SEQ ID NO: 22 - DNA, 26 bp, synthetic construct
  misc_feature 1..26: note = PCR Primer(DDX4) for Human
  source 1..26: mol_type = other DNA
taaacatgtctaagccccctaaagaa

SEQ ID NO: 23 - DNA, 22 bp, synthetic construct
  misc_feature 1..22: note = PCR Primer(SCP1) for Human
  source 1..22: mol_type = other DNA
aggccccttcatctctaacaac

SEQ ID NO: 24 - DNA, 22 bp, synthetic construct
  misc_feature 1..22: note = PCR Primer(SCP1) for Human
  source 1..22: mol_type = other DNA
tttagcaattacagcccaacgg

SEQ ID NO: 25 - DNA, 22 bp, synthetic construct
  misc_feature 1..22: note = PCR Primer(ZP3) for Human
  source 1..22: mol_type = other DNA
taacaaaggtgactgtggcact

SEQ ID NO: 26 - DNA, 22 bp, synthetic construct
  misc_feature 1..22: note = PCR Primer(ZP3) for Human
  source 1..22: mol_type = other DNA
ccactgctctacttcatggtca

SEQ ID NO: 27 - DNA, 26 bp, synthetic construct
  misc_feature 1..26: note = PCR Primer(FOXL2) for Human
  source 1..26: mol_type = other DNA
ccttcaaaaagctgtgttcagagtta

SEQ ID NO: 28 - DNA, 25 bp, synthetic construct
  misc_feature 1..25: note = PCR Primer(FOXL2) for Human
  source 1..25: mol_type = other DNA
ttcagatagggagagggtgaaactt